European Patent Application EP 4 137 503 A1, published February 22, 2023. Title: NOVEL CATHEPSIN INHIBITORS. Applicant: École Polytechnique Fédérale de Lausanne (EPFL). The sequence listing filed with the application follows.

SEQUENCE LISTING (2 sequences)

SEQ ID NO: 1 - DNA, 32 bp, Artificial Sequence
  CTSS_pHLsec_fw
gctgaaaccggtcagttgcataaagatcctac

SEQ ID NO: 2 - DNA, 35 bp, Artificial Sequence
  CTSS_pHLsec_rev
gtgcttggtaccgatttctgggtaagagggaaagc